European Patent Specification EP 3 501 605 B1, published June 28, 2023. Title: MRNA THERAPY FOR ARGININOSUCCINATE SYNTHETASE DEFICIENCY. Applicant: Translate Bio, Inc. Application Not yet assigned. The sequence listing filed with the application follows.

SEQUENCE LISTING (15 sequences)

SEQ ID NO: 1 - RNA, 1863 nt, Homo sapiens
gccggcgcgccccugggagggugagccggcgccgggcccaggcccggaccuggugggaggcggggggagguggggacgaggccuggggaggcgggccccgcccaucugcagguggcugugaacgcugagcggcuccaggcgggggccgggcccgggggcggggucuguggcgcgcguccccgccacguguccccggucaccggcccugcccccgggcccugugcuuauaaccugggaugggcaccccugccaguccugcucugccgccugccaccgcugcccgagcccgagugguucacugcacugugaaaacagauuccagacgccgggaacucacgccuccaaucccagacgcuauguccagcaaaggcuccgugguucuggccuacaguggcggccuggacaccucgugcauccucguguggcugaaggaacaaggcuaugacgucauugccuaucuggccaacauuggccagaaggaagacuucgaggaagccaggaagaaggcacugaagcuuggggccaaaaagguguucauugaggaugucagcagggaguuuguggaggaguucaucuggccggccauccaguccagcgcacuguaugaggaccgcuaccuccugggcaccucucuugccaggcccugcaucgcccgcaaacaaguggaaaucgcccagcgggagggggccaaguaugugucccacggcgccacaggaaaggggaacgaucagguccgguuugagcucagcugcuacucacuggccccccagauaaaggucauugcucccuggaggaugccugaauucuacaaccgguucaagggccgcaaugaccugauggaguacgcaaagcaacacgggauucccaucccggucacucccaagaacccguggagcauggaugagaaccucaugcacaucagcuacgaggcuggaauccuggagaaccccaagaaccaagcgccuccaggucucuacacgaagacccaggacccagccaaagcccccaacaccccugacauucucgagaucgaguucaaaaaaggggucccugugaaggugaccaacgucaaggauggcaccacccaccagaccuccuuggagcucuucauguaccugaacgaagucgcgggcaagcauggcgugggccguauugacaucguggagaaccgcuucauuggaaugaagucccgagguaucuacgagaccccagcaggcaccauccuuuaccaugcucauuuagacaucgaggccuucaccauggaccgggaagugcgcaaaaucaaacaaggccugggcuugaaauuugcugagcugguguauaccgguuucuggcacagcccugagugugaauuuguccgccacugcaucgccaagucccaggagcgaguggaagggaaagugcagguguccguccucaagggccagguguacauccucggccgggaguccccacugucucucuacaaugaggagcuggugagcaugaacgugcagggugauuaugagccaacugaugccaccggguucaucaacaucaauucccucaggcugaaggaauaucaucgucuccagagcaaggucacugccaaauagacccguguacaaugaggagcuggggccuccucaauuugcagaucccccaaguacaggcgcuaauuguugugauaauuuguaauugugacuuguucuccccggcuggcagcguaguggggcugccaggccccagcuuuguucccuggucccccugaagccugcaaacguugucaucgaagggaaggguggggggcagcugcgguggggagcuauaaaaaugacaauuaaaagagacacuagucuuuuauuucuaaaaaaaaaaaaaaaa

SEQ ID NO: 2 - protein, 412 aa, Homo sapiens
MSSKGSVVLAYSGGLDTSCILVWLKEQGYDVIAYLANIGQKEDFEEARKKALKLGAKKVFIEDVSREFVEEFIWPAIQSSALYEDRYLLGTSLARPCIARKQVEIAQREGAKYVSHGATGKGNDQVRFELSCYSLAPQIKVIAPWRMPEFYNRFKGRNDLMEYAKQHGIPIPVTPKNPWSMDENLMHISYEAGILENPKNQAPPGLYTKTQDPAKAPNTPDILEIEFKKGVPVKVTNVKDGTTHQTSLELFMYLNEVAGKHGVGRIDIVENRFIGMKSRGIYETPAGTILYHAHLDIEAFTMDREVRKIKQGLGLKFAELVYTGFWHSPECEFVRHCIAKSQERVEGKVQVSVLKGQVYILGRESPLSLYNEELVSMNVQGDYEPTDATGFININSLRLKEYHRLQSKVTAK

SEQ ID NO: 3 - RNA, 1239 nt, Artificial Sequence
  Description of Artificial Sequence: Synthetic polynucleotide
augagcagcaagggcagcguggugcuggccuacagcggcggccuggacaccagcugcauccugguguggcugaaggagcagggcuacgacgugaucgccuaccuggccaacaucggccagaaggaggacuucgaggaggcccgcaagaaggcccugaagcugggcgccaagaagguguucaucgaggacgugagccgcgaguucguggaggaguucaucuggcccgccauccagagcagcgcccuguacgaggaccgcuaccugcugggcaccagccuggcccgccccugcaucgcccgcaagcagguggagaucgcccagcgcgagggcgccaaguacgugagccacggcgccaccggcaagggcaacgaccaggugcgcuucgagcugagcugcuacagccuggccccccagaucaaggugaucgcccccuggcgcaugcccgaguucuacaaccgcuucaagggccgcaacgaccugauggaguacgccaagcagcacggcauccccauccccgugacccccaagaaccccuggagcauggacgagaaccugaugcacaucagcuacgaggccggcauccuggagaaccccaagaaccaggccccccccggccuguacaccaagacccaggaccccgccaaggcccccaacacccccgacauccuggagaucgaguucaagaagggcgugcccgugaaggugaccaacgugaaggacggcaccacccaccagaccagccuggagcuguucauguaccugaacgagguggccggcaagcacggcgugggccgcaucgacaucguggagaaccgcuucaucggcaugaagagccgcggcaucuacgagacccccgccggcaccauccuguaccacgcccaccuggacaucgaggccuucaccauggaccgcgaggugcgcaagaucaagcagggccugggccugaaguucgccgagcugguguacaccggcuucuggcacagccccgagugcgaguucgugcgccacugcaucgccaagagccaggagcgcguggagggcaaggugcaggugagcgugcugaagggccagguguacauccugggccgcgagagcccccugagccuguacaacgaggagcuggugagcaugaacgugcagggcgacuacgagcccaccgacgccaccggcuucaucaacaucaacagccugcgccugaaggaguaccaccgccugcagagcaaggugaccgccaaguga

SEQ ID NO: 4 - RNA, 140 nt, Artificial Sequence
  Description of Artificial Sequence: Synthetic polynucleotide
ggacagaucgccuggagacgccauccacgcuguuuugaccuccauagaagacaccgggaccgauccagccuccgcggccgggaacggugcauuggaacgcggauuccccgugccaagagugacucaccguccuugacacg

SEQ ID NO: 5 - RNA, 105 nt, Artificial Sequence
  Description of Artificial Sequence: Synthetic polynucleotide
cggguggcaucccugugaccccuccccagugccucuccuggcccuggaaguugccacuccagugcccaccagccuuguccuaauaaaauuaaguugcaucaagcu

SEQ ID NO: 6 - RNA, 105 nt, Artificial Sequence
  Description of Artificial Sequence: Synthetic polynucleotide
ggguggcaucccugugaccccuccccagugccucuccuggcccuggaaguugccacuccagugcccaccagccuuguccuaauaaaauuaaguugcaucaaagcu

SEQ ID NO: 7 - RNA, 1484 nt, Artificial Sequence
  Description of Artificial Sequence: Synthetic polynucleotide
ggacagaucgccuggagacgccauccacgcuguuuugaccuccauagaagacaccgggaccgauccagccuccgcggccgggaacggugcauuggaacgcggauuccccgugccaagagugacucaccguccuugacacgaugagcagcaagggcagcguggugcuggccuacagcggcggccuggacaccagcugcauccugguguggcugaaggagcagggcuacgacgugaucgccuaccuggccaacaucggccagaaggaggacuucgaggaggcccgcaagaaggcccugaagcugggcgccaagaagguguucaucgaggacgugagccgcgaguucguggaggaguucaucuggcccgccauccagagcagcgcccuguacgaggaccgcuaccugcugggcaccagccuggcccgccccugcaucgcccgcaagcagguggagaucgcccagcgcgagggcgccaaguacgugagccacggcgccaccggcaagggcaacgaccaggugcgcuucgagcugagcugcuacagccuggccccccagaucaaggugaucgcccccuggcgcaugcccgaguucuacaaccgcuucaagggccgcaacgaccugauggaguacgccaagcagcacggcauccccauccccgugacccccaagaaccccuggagcauggacgagaaccugaugcacaucagcuacgaggccggcauccuggagaaccccaagaaccaggccccccccggccuguacaccaagacccaggaccccgccaaggcccccaacacccccgacauccuggagaucgaguucaagaagggcgugcccgugaaggugaccaacgugaaggacggcaccacccaccagaccagccuggagcuguucauguaccugaacgagguggccggcaagcacggcgugggccgcaucgacaucguggagaaccgcuucaucggcaugaagagccgcggcaucuacgagacccccgccggcaccauccuguaccacgcccaccuggacaucgaggccuucaccauggaccgcgaggugcgcaagaucaagcagggccugggccugaaguucgccgagcugguguacaccggcuucuggcacagccccgagugcgaguucgugcgccacugcaucgccaagagccaggagcgcguggagggcaaggugcaggugagcgugcugaagggccagguguacauccugggccgcgagagcccccugagccuguacaacgaggagcuggugagcaugaacgugcagggcgacuacgagcccaccgacgccaccggcuucaucaacaucaacagccugcgccugaaggaguaccaccgccugcagagcaaggugaccgccaagugacggguggcaucccugugaccccuccccagugccucuccuggcccuggaaguugccacuccagugcccaccagccuuguccuaauaaaauuaaguugcaucaagcu

SEQ ID NO: 8 - RNA, 1484 nt, Artificial Sequence
  Description of Artificial Sequence: Synthetic polynucleotide
ggacagaucgccuggagacgccauccacgcuguuuugaccuccauagaagacaccgggaccgauccagccuccgcggccgggaacggugcauuggaacgcggauuccccgugccaagagugacucaccguccuugacacgaugagcagcaagggcagcguggugcuggccuacagcggcggccuggacaccagcugcauccugguguggcugaaggagcagggcuacgacgugaucgccuaccuggccaacaucggccagaaggaggacuucgaggaggcccgcaagaaggcccugaagcugggcgccaagaagguguucaucgaggacgugagccgcgaguucguggaggaguucaucuggcccgccauccagagcagcgcccuguacgaggaccgcuaccugcugggcaccagccuggcccgccccugcaucgcccgcaagcagguggagaucgcccagcgcgagggcgccaaguacgugagccacggcgccaccggcaagggcaacgaccaggugcgcuucgagcugagcugcuacagccuggccccccagaucaaggugaucgcccccuggcgcaugcccgaguucuacaaccgcuucaagggccgcaacgaccugauggaguacgccaagcagcacggcauccccauccccgugacccccaagaaccccuggagcauggacgagaaccugaugcacaucagcuacgaggccggcauccuggagaaccccaagaaccaggccccccccggccuguacaccaagacccaggaccccgccaaggcccccaacacccccgacauccuggagaucgaguucaagaagggcgugcccgugaaggugaccaacgugaaggacggcaccacccaccagaccagccuggagcuguucauguaccugaacgagguggccggcaagcacggcgugggccgcaucgacaucguggagaaccgcuucaucggcaugaagagccgcggcaucuacgagacccccgccggcaccauccuguaccacgcccaccuggacaucgaggccuucaccauggaccgcgaggugcgcaagaucaagcagggccugggccugaaguucgccgagcugguguacaccggcuucuggcacagccccgagugcgaguucgugcgccacugcaucgccaagagccaggagcgcguggagggcaaggugcaggugagcgugcugaagggccagguguacauccugggccgcgagagcccccugagccuguacaacgaggagcuggugagcaugaacgugcagggcgacuacgagcccaccgacgccaccggcuucaucaacaucaacagccugcgccugaaggaguaccaccgccugcagagcaaggugaccgccaagugaggguggcaucccugugaccccuccccagugccucuccuggcccuggaaguugccacuccagugcccaccagccuuguccuaauaaaauuaaguugcaucaaagcu

SEQ ID NO: 9 - DNA, 300 bp, Artificial Sequence
  Description of Artificial Sequence: Synthetic polynucleotide
  misc_feature (1)..(300): This sequence may encompass 10-300 nucleotides
  See specification as filed for detailed description of substitutions and preferred embodiments
aaaaaaaaaaaaaaaaaaaaaaaaaaaaaaaaaaaaaaaaaaaaaaaaaaaaaaaaaaaaaaaaaaaaaaaaaaaaaaaaaaaaaaaaaaaaaaaaaaaaaaaaaaaaaaaaaaaaaaaaaaaaaaaaaaaaaaaaaaaaaaaaaaaaaaaaaaaaaaaaaaaaaaaaaaaaaaaaaaaaaaaaaaaaaaaaaaaaaaaaaaaaaaaaaaaaaaaaaaaaaaaaaaaaaaaaaaaaaaaaaaaaaaaaaaaaaaaaaaaaaaaaaaaaaaaaaaaaaaaaaaaaaaaaaaaaaaaaaaaa

SEQ ID NO: 10 - DNA, 200 bp, Artificial Sequence
  Description of Artificial Sequence: Synthetic polynucleotide
  misc_feature (1)..(200): This sequence may encompass 10-200 nucleotides
  See specification as filed for detailed description of substitutions and preferred embodiments
cccccccccccccccccccccccccccccccccccccccccccccccccccccccccccccccccccccccccccccccccccccccccccccccccccccccccccccccccccccccccccccccccccccccccccccccccccccccccccccccccccccccccccccccccccccccccccccccccccccccc

SEQ ID NO: 11 - DNA, 500 bp, Artificial Sequence
  Description of Artificial Sequence: Synthetic polynucleotide
  misc_feature (1)..(500): This sequence may encompass 10-500 nucleotides
  See specification as filed for detailed description of substitutions and preferred embodiments
aaaaaaaaaaaaaaaaaaaaaaaaaaaaaaaaaaaaaaaaaaaaaaaaaaaaaaaaaaaaaaaaaaaaaaaaaaaaaaaaaaaaaaaaaaaaaaaaaaaaaaaaaaaaaaaaaaaaaaaaaaaaaaaaaaaaaaaaaaaaaaaaaaaaaaaaaaaaaaaaaaaaaaaaaaaaaaaaaaaaaaaaaaaaaaaaaaaaaaaaaaaaaaaaaaaaaaaaaaaaaaaaaaaaaaaaaaaaaaaaaaaaaaaaaaaaaaaaaaaaaaaaaaaaaaaaaaaaaaaaaaaaaaaaaaaaaaaaaaaaaaaaaaaaaaaaaaaaaaaaaaaaaaaaaaaaaaaaaaaaaaaaaaaaaaaaaaaaaaaaaaaaaaaaaaaaaaaaaaaaaaaaaaaaaaaaaaaaaaaaaaaaaaaaaaaaaaaaaaaaaaaaaaaaaaaaaaaaaaaaaaaaaaaaaaaaaaaaaaaaaaaaaaaaaaaaaaaaaaaaaaaaaaaaaaaaaaaaaaaa

SEQ ID NO: 12 - DNA, 250 bp, Artificial Sequence
  Description of Artificial Sequence: Synthetic polynucleotide
  See specification as filed for detailed description of substitutions and preferred embodiments
aaaaaaaaaaaaaaaaaaaaaaaaaaaaaaaaaaaaaaaaaaaaaaaaaaaaaaaaaaaaaaaaaaaaaaaaaaaaaaaaaaaaaaaaaaaaaaaaaaaaaaaaaaaaaaaaaaaaaaaaaaaaaaaaaaaaaaaaaaaaaaaaaaaaaaaaaaaaaaaaaaaaaaaaaaaaaaaaaaaaaaaaaaaaaaaaaaaaaaaaaaaaaaaaaaaaaaaaaaaaaaaaaaaaaaaaaaaaaaaaaaaaaaaaaa

SEQ ID NO: 13 - RNA, 1239 nt, Artificial Sequence
  Description of Artificial Sequence: Synthetic polynucleotide
augagcucaaagggaucuguggugcuggcauacucggggggauuggacacuucaugcauacuugucugguugaaggaacagggcuacgacgugaucgccuaccuggcuaacaucggucaaaaggaggacuucgaggaggcccggaagaaggcccugaagcugggcgcgaagaaaguguucaucgaggacgugucccgggaauuuguggaagaguucaucuggcccgccauccaaagcagcgcacuguacgaggauagauaccuccucggaacaucccuugcccggccauguauugccaggaaacagguggaaaucgcccagcgggaaggagccaaauacgugucccacggggcgaccggaaaggggaacgaccaagugcgcuucgagcugucgugcuacucccuggcaccgcagauuaaggucaucgcgccguggagaaugccugaauucuacaaccgcuucaagggccgcaacgaucugauggaauacgccaagcagcacggcaucccgauccccgugaccccuaagaacccuuggucaauggacgagaaucugaugcacaucagcuacgaagcgggcauccuggagaaccccaagaaucaagcuccgcccggacuguacacuaagacucaggaucccgcuaaggcgcccaacacuccugauauuuuggaaaucgaauucaagaagggugucccagugaaggucaccaacgugaaggacggcacuacccaccagaccucgcuggaacuguuuauguaucugaacgagguggccggcaaacauggagucggcagaaucgauauuguggagaaccgcuuuauuggcaugaaguccagggggaucuaugaaaccccggccggaaccauccucuaccacgcccaucucgacauugaagcguucaccauggaccgcgagguccgcaagauuaagcagggccugggacucaaguucgccgagcucguguacaccgguuucuggcauuccccggaaugcgaauucgugcgacacugcauugccaagagccaggagcggguggaaggaaagguccagguguccgugcugaagggucaaguguacauccuggggcgggaguccccucuuucccuguacaacgaagaacuggugucgaugaacgugcagggagacuacgagccgaccgacgccacggguuucauuaacaucaauucccugagacugaaggaguaccaccggcuccaguccaaagucaccgcuaaguga

SEQ ID NO: 14 - RNA, 1239 nt, Artificial Sequence
  Description of Artificial Sequence: Synthetic polynucleotide
augagcucaaaaggaucgguggugcuggcauacucgggaggauuggacacuucauguauucuugucuggcucaaggaacagggcuacgacgucauugccuaccuggccaacaucggucagaaagaggacuucgaggaagccagaaagaaggcccugaagcugggagccaagaagguguucaucgaggacgugucccgcgaauuuguggaagaauucaucuggccugccauucaauccuccgcgcucuacgaggaucgguaccuucugggaacuuccuuggcucgcccgugcaucgcccggaaacaaguggagauugcacagcgggaaggagcuaaguacgugucccacggggccacuggaaagggcaacgaucaagugcgcuucgagcuguccugcuacucccuggcgccacagaucaaggucaucgcgccguggcggaugcccgaguucuauaaccgcuucaagggacggaacgaucugauggaguacgccaagcagcacggcauuccgauacccgugacccccaagaacccuuggagcauggacgagaaccugaugcauaucucuuacgaagccgggauucucgaaaacccuaagaaucaggcgccgccuggccuguacaccaaaacccaggaccccgccaaggcgccgaacacgcccgacauccucgaaaucgaguucaagaagggggugccagugaaggucaccaacgugaaggacggaaccacccaucagaccucacuggaacucuucauguaccucaacgaggucgcagggaagcacggcguggggagaaucgacaucguggaaaacagguucaucggcaugaagucccggggaaucuacgaaacacccgccgggacuauccucuaccacgcccaccuggacauugaggccuucaccauggauagagaagugcgcaagauuaagcagggucugggucugaaguucgccgaguuggucuacaccggauucuggcauuccccugaaugcgaauucgugcgccacugcauugccaagagccaggaaagaguggagggcaaaguccaagugucggugcugaagggccaaguguacauccugggaagggaaagcccgcucucccuguacaacgaggaacuggugucgaugaacguccagggcgauuaugagccgacugacgccacugguuuuaucaauaucaacagccugcgacugaaggaguaccaccggcugcaguccaaggucaccgcuaaguag

SEQ ID NO: 15 - RNA, 1239 nt, Artificial Sequence
  Description of Artificial Sequence: Synthetic polynucleotide
augagcucgaaaggauccgugguuuuggcauacuccgguggacuugacacuucaugcauuuugguuuggcucaaagaacagggcuacgaugugaucgccuaccuggcgaacaucggacagaaagaggacuuugaagaggcccgcaagaaggcacugaagcugggugccaagaaaguguuuaucgaggaugugucgagagaauucguggaagaauucauuuggccagccauucaaagcuccgcgcuguacgaggacagauaccuccucggcaccucacuggcccgcccuugcaucgcgcgcaaacaggucgagaucgcucaaagagaaggagcuaaauacgugucacacggcgccaccggaaagggaaaugaccaaguccgcuucgagcugucuugcuacucacucgcuccgcaaaucaaggucaucgcaccguggaggaugcccgaguucuacaaccgguucaaggggcggaacgaccugauggaguacgcgaagcagcacgguaucccgaucccugucaccccaaagaaccccuggagcauggacgaaaaucugaugcacaucagcuacgaagcaggaauccuggagaacccgaaaaaucaagcaccuccuggacuguacacuaagacccaggacccagccaaggccccgaauaccccggacaucuuggaaaucgaguucaagaagggggugccagugaagguuaccaaugucaaggaugggaccacucaccaaacuagccuggaacuguucauguaccugaacgaaguggcuggaaaacauggcgugggaagaaucgauaucguggagaaccgcuucaucggcaugaagucaaggggaaucuacgaaacuccggccgggacgauacuguaucaugcgcaucucgacauugaagccuuuacuauggaucgggaaguccgaaagaucaaacagggcuugggccucaaguuugccgagcugguguacacgggauucuggcacucgccggaaugcgaauucgugcgccacuguauugcgaagucccaggagcgcguggaagggaagguccaagucuccgugcucaaaggacaggucuacauccuuggacgggagucgccccugucgcucuacaacgaagaacuggugucgaugaacgugcagggagacuaugaaccaacggaugcuacugguuucaucaacaucaauucgcugcggcuuaaggaguaccaucggcugcaguccaaggucaccgcgaaguag